European Patent Specification EP 3 600 405 B1, published August 20, 2025. Title: GLYCAN-MASKED ENGINEERED OUTER DOMAINS OF HIV-1 GP120  AND THEIR USE. Applicant: The United States of America, as Represented by the Secretary, Department of Health and human Services. The sequence listing filed with the application follows.

SEQUENCE LISTING (113 sequences)

SEQ ID NO: 1 - protein, 172 aa, Artificial Sequence
  recombinant gp120 protein
DTITLPCRPAPPPHCSSNITGLILTRQGGYSNDNTVIFRPSGGDWRDIARCQIAGTVVSTQLFLNGSLAEEEVVIRSEDWRDNAKSICVQLNTSVEINCTGAGHCNISRAKWNNTLKQIASKLREQYGNKTIIFKPSSGGDPEFVNHSFNCGGEFFYCDSTQLFNSTWFNST

SEQ ID NO: 2 - protein, 172 aa, Artificial Sequence
  recombinant gp120 protein
DTITLPCRPAPPPHCSSNITGLILTRQGGYSNDNTVIFRPSGGDWRDIARCQIAGTVVSTQLFLNGSLANGTVVIRSEDWRDNAKSICVQLNTSVEINCTGAGHCNISRAKWNNTLKQIASKLREQYGNKTIIFKPSSGGDPEFVNHSFNCGGEFFYCDSTQLFNSTWFNST

SEQ ID NO: 3 - protein, 172 aa, Artificial Sequence
  recombinant gp120 protein
DTITLPCRPAPPPNCTSNITGLILTRQGGYSNDNTVIFRPSGGDWRDIARCQIAGTVVSTQLFLNGSLAEEEVVIRSEDWRDNAKSICVQLNTSVEINCTGAGHCNISRAKWNNTLKQIASKLREQYGNKTIIFKPSSGGDPEFVNHSFNCGGEFFYCDSTQLFNSTWFNST

SEQ ID NO: 4 - protein, 172 aa, Artificial Sequence
  recombinant gp120 protein
DTITLPCRPAPPPHCSSNITGLILTRQGGYSNDNTVIFRPSGGDWRDIARCNITGTVVSTQLFLNGSLAEEEVVIRSEDWRDNAKSICVQLNTSVEINCTGAGHCNISRAKWNNTLKQIASKLREQYGNKTIIFKPSSGGDPEFVNHSFNCGGEFFYCDSTQLFNSTWFNST

SEQ ID NO: 5 - protein, 172 aa, Artificial Sequence
  recombinant gp120 protein
DTITLPCRPAPPPHCSSNITGLILTRQGGYSNDNTVIFRPSGGDWRDIARCQIAGNVTSTQLFLNGSLAEEEVVIRSEDWRDNAKSICVQLNTSVEINCTGAGHCNISRAKWNNTLKQIASKLREQYGNKTIIFKPSSGGDPEFVNHSFNCGGEFFYCDSTQLFNSTWFNST

SEQ ID NO: 6 - protein, 172 aa, Artificial Sequence
  recombinant gp120 protein
DTITLPCRPAPPPHCSSNITGLILTRQGGYSNDNTVIFRPSGGDWRDIARCQIAGTVVSTQLFLNGSLAEEEVVIRSEDWRDNAKSICVQLNTSVEINCTGAGHCNISRAKWNNTLKQIASKLREQYGNKTIIFKPSSGGDPEFVNHSFNCTGEFFYCDSTQLFNSTWFNST

SEQ ID NO: 7 - protein, 172 aa, Artificial Sequence
  recombinant gp120 protein
DTITLPCRPAPPPHCSSNITGLILTRQGGYSNDNTVIFRPSGGDWRDIARCQIAGTVVSTQLFLNGSLAEEEVVIRSEDWRDNAKSICVQLNTSVEINCTGAGHCNISRAKWNNTLKQIASKLREQYGNKTIIFKPSSGGDPEFVNHSFNCGNVTFYCDSTQLFNSTWFNST

SEQ ID NO: 8 - protein, 172 aa, Artificial Sequence
  recombinant gp120 protein
DNITLPCRPAPPPHCSSNITGLILTRQGGYSNDNTVIFRPSGGDWRDIARCQIAGTVVSTQLFLNGSLAEEEVVIRSEDWRDNAKSICVQLNTSVEINCTGAGHCNISRAKWNNTLKQIASKLREQYGNKTIIFKPSSGGDPEFVNHSFNCGGEFFYCDSTQLFNSTWFNST

SEQ ID NO: 9 - protein, 172 aa, Artificial Sequence
  recombinant gp120 protein
DTITLPCRPAPPPHCSSNITGLILTRQGGYSNDNTVIFRPSGGDWRDIARCQIAGTVVSTQLFLNGSLAEEEVVIRSEDWRDNAKSICVQLNTSVEINCTGAGHCNISRAKWNNTLKQIANKTREQYGNKTIIFKPSSGGDPEFVNHSFNCGGEFFYCDSTQLFNSTWFNST

SEQ ID NO: 10 - protein, 172 aa, Artificial Sequence
  recombinant gp120 protein
DTITLPCRPAPPPHCSSNITGLILTRQGGYSNDNTVIFRPSGGDWRDIARCQIAGTVVSTQLFLNGSLAEEEVVIRSEDWRDNAKSICVQLNTSVEINCTGNGTCNISRAKWNNTLKQIASKLREQYGNKTIIFKPSSGGDPEFVNHSFNCGGEFFYCDSTQLFNSTWFNST

SEQ ID NO: 11 - protein, 173 aa, Artificial Sequence
  recombinant gp120 protein
DTITLPCNGTGPPPHCSSNITGLILTRQGGYSNDNTVIFRPSGGDWRDIARCQIAGTVVSTQLFLNGSLAEEEVVIRSEDWRDNAKSICVQLNTSVEINCTGAGHCNISRAKWNNTLKQIASKLREQYGNKTIIFKPSSGGDPEFVNHSFNCGGEFFYCDSTQLFNSTWFNST

SEQ ID NO: 12 - protein, 172 aa, Artificial Sequence
  recombinant gp120 protein
DTITLPCRPAPPPHCSSNITGLILTRQGGYSNDNTVIFRPSGGDWRDIARCQIAGTVVSTQLFLNGSLAEEEVVIRSEDWRDNAKSICVQLNTSVEINCTGAGHCNISRAKWNNTLKQIASKLREQYGNKTIIFKPSSGGDPEFVNHSFNCGGEFFYCNSTQLFNSTWFNST

SEQ ID NO: 13 - protein, 172 aa, Artificial Sequence
  recombinant gp120 protein
DTITLPCRPAPPPNCTSNITGLILTRQGGYSNDNTVIFRPSGGDWRDIARCQIAGNVTSTQLFLNGSLAGNGTVIRSEDWRDNAKSICVQLNTSVEINCTGAGHCNISRAKWNNTLKQIASKLREQYGNKTIIFKPSSGGDPEFVNHSFNCGGEFFYCDSTQLFNSTWFNST

SEQ ID NO: 14 - protein, 172 aa, Artificial Sequence
  recombinant gp120 protein
DTITLPCRPAPPPNCTSNITGLILTRQGGYSNDNTVIFRPSGGDWRDIARCNITGTVVSTQLFLNGSLAGNGTVIRSEDWRDNAKSICVQLNTSVEINCTGAGHCNISRAKWNNTLKQIASKLREQYGNKTIIFKPSSGGDPEFVNHSFNCGGEFFYCDSTQLFNSTWFNST

SEQ ID NO: 15 - protein, 173 aa, Artificial Sequence
  recombinant gp120 protein
DTITLPCNGTGPPPHCSSNITGLILTRQGGYSNDNTVIFRPSGGDWRDIARCNITGTVVSTQLFLNGSLAGNGTVIRSEDWRDNAKSICVQLNTSVEINCTGAGHCNISRAKWNNTLKQIASKLREQYGNKTIIFKPSSGGDPEFVNHSFNCGGEFFYCDSTQLFNSTWFNST

SEQ ID NO: 16 - protein, 172 aa, Artificial Sequence
  recombinant gp120 protein
DTITLPCRPAPPPNCTSNITGLILTRQGGYSNDNTVIFRPSGGDWRDIARCNITGTVVSTQLFLNGSLAGNGTVIRSEDWRDNAKSICVQLNTSVEINCTGNGTCNISRAKWNNTLKQIASKLREQYGNKTIIFKPSSGGDPEFVNHSFNCGNVTFYCDSTQLFNSTWFNST

SEQ ID NO: 17 - protein, 172 aa, Artificial Sequence
  recombinant gp120 protein
DTITLPCRPAPPPNCTSNITGLILTRQGGYSNDNTVIFRPSGGDWRDIARCNITGTVVSTQLFLNGSLAGNGTVIRSEDWRDNAKSICVQLNTSVEINCTGNGTCNISRAKWNNTLKQIASKLREQYGNKTIIFKPSSGGDPEFVNHSFNCTGEFFYCDSTQLFNSTWFNST

SEQ ID NO: 18 - protein, 172 aa, Artificial Sequence
  recombinant gp120 protein
DNITLPCRPAPPPNCTSNITGLILTRQGGYSNDNTVIFRPSGGDWRDIARCNITGNVTSTQLFLNGSLAGNGTVIRSEDWRDNAKSICVQLNTSVEINCTGAGHCNISRAKWNNTLKQIASKLREQYGNKTIIFKPSSGGDPEFVNHSFNCTGEFFYCDSTQLFNSTWFNST

SEQ ID NO: 19 - protein, 172 aa, Artificial Sequence
  recombinant gp120 protein
DNITLPCRPAPPPNCTSNITGLILTRQGGYSNDNTVIFRPSGGDWRDIARCQIAGTVVSTQLFLNGSLANGTVVIRSEDWRDNAKSICVQLNTSVEINCTGNGTCNISRAKWNNTLKQIASKLREQYGNKTIIFKPSSGGDPEFVNHSFNCTGEFFYCDSTQLFNSTWFNST

SEQ ID NO: 20 - protein, 172 aa, Artificial Sequence
  recombinant gp120 protein
DNITLPCRPAPPPHCSSNITGLILTRQGGYSNDNTVIFRPSGGDWRDIARCQIAGTVVSTQLFLNGSLAGNGTVIRSEDWRDNAKSICVQLNTSVEINCTGAGHCNISRAKWNNTLKQIANKTREQYGNKTIIFKPSSGGDPEFVNHSFNCGGEFFYCDSTQLFNSTWFNST

SEQ ID NO: 21 - protein, 173 aa, Artificial Sequence
  recombinant gp120 protein
DTITLPCNGTGPPPNCTSNITGLILTRQGGYSNDNTVIFRPSGGDWRDIARCNITGTVVSTQLFLNGSLANGTVVIRSEDWRDNAKSICVQLNTSVEINCTGNGTCNISRAKWNNTLKQIASKLREQYGNKTIIFKPSSGGDPEFVNHSFNCGNVTFYCDSTQLFNSTWFNST

SEQ ID NO: 22 - protein, 172 aa, Artificial Sequence
  recombinant gp120 protein
DNITLPCRPAPPPNCTSNITGLILTRQGGYSNDNTVIFRPSGGDWRDIARCNITGNVTSTQLFLNGSLAGGEVNGTSEDWRDNAKSICVQLNTSVEINCTGAGHCNISRAKWNNTLKQIASKLREQYGNKTIIFKPSSGGDPEFVNHSFNCGNVTFYCDSTQLFNSTWFNST

SEQ ID NO: 23 - protein, 172 aa, Artificial Sequence
  recombinant gp120 protein
DTITLPCRPAPPPHCSSNITGLILTRQGGYSNDNTVIFRPSGGDWRDIARCQIAGTVVSTQLFLNGSLAGGEVNGTSEDWRDNAKSICVQLNTSVEINCTGAGHCNISRAKWNNTLKQIASKLREQYGNKTIIFKPSSGGDPEFVNHSFNCGGEFFYCDSTQLFNSTWFNST

SEQ ID NO: 24 - protein, 172 aa, Artificial Sequence
  recombinant gp120 protein
DTITLPCRPAPPPHCSSNITGLILTRQGGYSNDNTVIFRPSGGDWRDIARCQIAGTVVSTQLFLNGSLAGNGTVIRSEDWRDNAKSICVNLTTSVEINCTGAGHCNISRAKWNNTLKQIASKLREQYGNKTIIFKPSSGGDPEFVNHSFNCGGEFFYCDSTQLFNSTWFNST

SEQ ID NO: 25 - protein, 173 aa, Artificial Sequence
  recombinant gp120 protein
DTITLPCNGTGPPPHCSSNITGLILTRQGGYSNDNTVIFRPSGGDWRDIARCQIAGTVVSTQLFLNGSLAGNGTVIRSEDWRDNAKSICVQLNTSVEINCTGAGHCNISRAKWNNTLKQIASKLREQYGNKTIIFKPSSGGDPEFVNHSFNCGGEFFYCDSTQLFNSTWFNST

SEQ ID NO: 26 - protein, 172 aa, Artificial Sequence
  recombinant gp120 protein
DTITLPCRPAPPPHCSSNITGLILTRQGGYSNDNTVIFRPSGGDWRDIARCQIAGTVVSTQLFLNGSLAGNGTVIRSEDWRDNAKSICVQLNTSVEINCTGNGTCNISRAKWNNTLKQIASKLREQYGNKTIIFKPSSGGDPEFVNHSFNCGNVTFYCDSTQLFNSTWFNST

SEQ ID NO: 27 - protein, 172 aa, Artificial Sequence
  recombinant gp120 protein
DTITLPCRPAPPPHCSSNITGLILTRQGGYSNDNTVIFRPSGGDWRDIARCQIAGTVVSTQLFLNGSLAGNGTVIRSEDWRDNAKSICVNLTTSVEINCTGNGTCNISRAKWNNTLKQIASKLREQYGNKTIIFKPSSGGDPEFVNHSFNCGNVTFYCDSTQLFNSTWFNST

SEQ ID NO: 28 - protein, 172 aa, Artificial Sequence
  recombinant gp120 protein
DTITLPCRPAPPPHCSSNITGLILTRQGGYSNDNTVIFRPSGGDWRDIARCNITGTVVSTQLFLNGSLAGNGTVIRSEDWRDNAKSICVQLNTSVEINCTGNGTCNISRAKWNNTLKQIASKLREQYGNKTIIFKPSSGGDPEFVNHSFNCGNVTFYCDSTQLFNSTWFNST

SEQ ID NO: 29 - protein, 172 aa, Artificial Sequence
  recombinant gp120 protein
DTITLPCRPAPPPHCSSNITGLILTRQGGYSNDNTVIFRPSGGDWRDIARCQIAGNVTSTQLFLNGSLAGNGTVIRSEDWRDNAKSICVQLNTSVEINCTGNGTCNISRAKWNNTLKQIASKLREQYGNKTIIFKPSSGGDPEFVNHSFNCGNVTFYCDSTQLFNSTWFNST

SEQ ID NO: 30 - protein, 172 aa, Artificial Sequence
  recombinant gp120 protein
DNITLPCRPAPPPHCSSNITGLILTRQGGYSNDNTVIFRPSGGDWRDIARCQIAGTVVSTQLFLNGSLAGNGTVIRSEDWRDNAKSICVQLNTSVEINCTGNGTCNISRAKWNNTLKQIASKLREQYGNKTIIFKPSSGGDPEFVNHSFNCGNVTFYCDSTQLFNSTWFNST

SEQ ID NO: 31 - protein, 172 aa, Artificial Sequence
  recombinant gp120 protein
DTITLPCRPAPPPHCSSNITGLILTRQGGYSNDNTVIFRPSGGDWRDIARCQIAGTVVSTQLFLNGSLAGNGTVIRSEDWRDNAKSICVQLNTSVEINCTGNGTCNISRAKWNNTLKQIANKTREQYGNKTIIFKPSSGGDPEFVNHSFNCGNVTFYCDSTQLFNSTWFNST

SEQ ID NO: 32 - protein, 172 aa, Artificial Sequence
  recombinant gp120 protein
DTITLPCRPAPPPHCSSNITGLILTRQGGYSNDNTVIFRPSGGDWRDIARCQIAGTVVSTQLFLNGSLAGNGTVIRSEDWRDNAKSICVQLNTSVEINCTGNGTCNISRAKWNNTLKQIASKLREQYGNKTIIFKPSSGGDPEFVNHSFNCGNVTFYCNSTQLFNSTWFNST

SEQ ID NO: 33 - protein, 173 aa, Artificial Sequence
  recombinant gp120 protein
DTITLPCNGTGPPPHCSSNITGLILTRQGGYSNDNTVIFRPSGGDWRDIARCNITGTVVSTQLFLNGSLAGNGTVIRSEDWRDNAKSICVQLNTSVEINCTGAGHCNISRAKWNNTLKQIASKLREQYGNKTIIFKPSSGGDPEFVNHSFNCGNVTFYCDSTQLFNSTWFNST

SEQ ID NO: 34 - protein, 173 aa, Artificial Sequence
  recombinant gp120 protein
DNITLPCNGTGPPPHCSSNITGLILTRQGGYSNDNTVIFRPSGGDWRDIARCNITGTVVSTQLFLNGSLAGNGTVIRSEDWRDNAKSICVQLNTSVEINCTGAGHCNISRAKWNNTLKQIASKLREQYGNKTIIFKPSSGGDPEFVNHSFNCGNVTFYCDSTQLFNSTWFNST

SEQ ID NO: 35 - protein, 173 aa, Artificial Sequence
  recombinant gp120 protein
DNITLPCNGTGPPPHCSSNITGLILTRQGGYSNDNTVIFRPSGGDWRDIARCNITGTVVSTQLFLNGSLAGNGTVIRSEDWRDNAKSICVQLNTSVEINCTGAGHCNISRAKWNNTLKQIASKLREQYGNKTIIFKPSSGGDPEFVNHSFNCGGEFFYCNSTQLFNSTWFNST

SEQ ID NO: 36 - protein, 173 aa, Artificial Sequence
  recombinant gp120 protein
DTITLPCNGTGPPPHCSSNITGLILTRQGGYSNDNTVIFRPSGGDWRDIARCNITGTVVSTQLFLNGSLAGNGTVIRSEDWRDNAKSICVQLNTSVEINCTGNGTCNISRAKWNNTLKQIASKLREQYGNKTIIFKPSSGGDPEFVNHSFNCGNVTFYCDSTQLFNSTWFNST

SEQ ID NO: 37 - protein, 173 aa, Artificial Sequence
  recombinant gp120 protein
DTITLPCNGTGPPPHCSSNITGLILTRQGGYSNDNTVIFRPSGGDWRDIARCNITGTVVSTQLFLNGSLAGNGTVIRSEDWRDNAKSICVQLNTSVEINCTGAGHCNISRAKWNNTLKQIASKLREQYGNKTIIFKPSSGGDPEFVNHSFNCGNVTFYCNSTQLFNSTWFNST

SEQ ID NO: 38 - protein, 173 aa, Artificial Sequence
  recombinant gp120 protein
DTITLPCNGTGPPPHCSSNITGLILTRQGGYSNDNTVIFRPSGGDWRDIARCNITGTVVSTQLFLNGSLAGNGTVIRSEDWRDNAKSICVQLNTSVEINCTGNGTCNISRAKWNNTLKQIASKLREQYGNKTIIFKPSSGGDPEFVNHSFNCGGEFFYCNSTQLFNSTWFNST

SEQ ID NO: 39 - protein, 173 aa, Artificial Sequence
  recombinant gp120 protein
DTITLPCNGTGPPPHCSSNITGLILTRQGGYSNDNTVIFRPSGGDWRDIARCNITGTVVSTQLFLNGSLAGNGTVIRSEDWRDNAKSICVNLTTSVEINCTGAGHCNISRAKWNNTLKQIASKLREQYGNKTIIFKPSSGGDPEFVNHSFNCGGEFFYCDSTQLFNSTWFNST

SEQ ID NO: 40 - protein, 173 aa, Artificial Sequence
  recombinant gp120 protein
DTITLPCNGTGPPPHCSSNITGLILTRQGGYSNDNTVIFRPSGGDWRNLARCNITGTVVSTQLFLNGSLAGNGTVIRSEDWRDNAKSICVQLNTSVEINCTGAGHCNISRAKWNNTLKQIASKLREQYGNKTIIFKPSSGGDPEFVNHSFNCGNVTFYCDSTQLFNSTWFNST

SEQ ID NO: 41 - protein, 173 aa, Artificial Sequence
  recombinant gp120 protein
DTITLPCNGTGPPPHCSSNITGLILTRQGGYSNDNTVIFRPSGGDWRNLARCNITGTVVSTQLFLNGSLAGNGTVIRSEDWRDNAKSICVQLNTSVEINCTGAGHCNISRAKWNNTLKQIASKLREQYGNKTIIFKPSSGGDPEFVNHSFNCGNVTFYCNSTQLFNSTWFNST

SEQ ID NO: 42 - protein, 173 aa, Artificial Sequence
  recombinant gp120 protein
DTITLPCNGTGPPPHCSSNITGLILTRQGGYSNDNTVIFRPSGGDWRDIARCNITGTVVSTQLFLNGSLAGNGTVIRSENFTDNAKSICVQLNTSVEINCTGAGHCNISRAKWNNTLKQIASKLREQYGNKTIIFKPSSGGDPEFVNHSFNCGGEFFYCDSTQLFNSTWFNST

SEQ ID NO: 43 - protein, 173 aa, Artificial Sequence
  recombinant gp120 protein
DTITLPCNGTGPPPHCSSNITGLILTRQGGYSNNGTVIFRPSGGDWRDIARCNITGTVVSTQLFLNGSLAGNGTVIRSENFTDNAKSICVQLNTSVEINCTGAGHCNISRAKWNNTLKQIASKLREQYGNKTIIFKPSSGGDPEFVNHSFNCGGEFFYCDSTQLFNSTWFNST

SEQ ID NO: 44 - protein, 172 aa, Artificial Sequence
  recombinant gp120 protein
DTITLPCRPAPPPNCTSNITGLILTRQGGYSNDNTVIFRPSGGDWRDIARCNITGTVVSTQLFLNGSLAGNGTVIRSENFTDNAKSICVQLNTSVEINCTGNGTCNISRAKWNNTLKQIASKLREQYGNKTIIFKPSSGGDPEFVNHSFNCGNVTFYCDSTQLFNSTWFNST

SEQ ID NO: 45 - protein, 173 aa, Artificial Sequence
  recombinant gp120 protein
DTITLPCNGTGPPPHCSSNITGLILTRQGGYSNDNTVIFRPSGGDWRNLARCNITGTVVSTQLFLNGSLAGNGTVIRSENFTDNAKSICVQLNTSVEINCTGAGHCNISRAKWNNTLKQIASKLREQYGNKTIIFKPSSGGDPEFVNHSFNCGNVTFYCDSTQLFNSTWFNST

SEQ ID NO: 46 - protein, 172 aa, Artificial Sequence
  recombinant gp120 protein
DNITLPCRPAPPPHCSSNITGLILTRQGGYSNDNTVIFRPSGGDWRDIARCQIAGTVVSTQLFLNGSLAGNGTVIRSENFTDNAKSICVQLNTSVEINCTGNGTCNISRAKWNNTLKQIASKLREQYGNKTIIFKPSSGGDPEFVNHSFNCGNVTFYCDSTQLFNSTWFNST

SEQ ID NO: 47 - protein, 172 aa, Artificial Sequence
  recombinant gp120 protein
DTITLPCRPAPPPHCSSNITGLILTRQGGYSNDNTVIFRPSGGDWRDIARCNITGTVVSTQLFLNGSLAGNGTVIRSENFTDNAKSICVQLNTSVEINCTGNGTCNISRAKWNNTLKQIASKLREQYGNKTIIFKPSSGGDPEFVNHSFNCGNVTFYCDSTQLFNSTWFNST

SEQ ID NO: 48 - protein, 173 aa, Artificial Sequence
  recombinant gp120 protein
DTITLPCNGTGPPPHCSSNITGLILTRQGGYSNDNTVIFRPSGGDWRDIARCNITGTVVSTQLFLNGSLAGNGTVIRSENFTDNAKSICVQLNTSVEINCTGAGHCNISRAKWNNTLKQIASKLREQYGNKTIIFKPSSGGDPEFVNHSFNCGNVTFYCNSTQLFNSTWFNST

SEQ ID NO: 49 - protein, 173 aa, Artificial Sequence
  Signal peptide
MGWSCIILFLVATATGVHSMQIYEGKLTAEGLRFGIVASRFNHALVDRLVEGAIDAIVRHGGREEDITLVRVPGSWEIPVAAGELARKEDIDAVIAIGVLIRGATPHFDYIASEVSKGLADLSLELRKPITFGVITADTLEQAIERAGTKHGNKGWEAALSAIEMANLFKSLR

SEQ ID NO: 50 - protein, 15 aa, Artificial Sequence
  Peptide linker
GGSGGSGGSGGSGGG

SEQ ID NO: 51 - protein, 361 aa, Artificial Sequence
  recombinant gp120 lumazine synthase fusion protein
MGWSCIILFLVATATGVHSMQIYEGKLTAEGLRFGIVASRFNHALVDRLVEGAIDAIVRHGGREEDITLVRVPGSWEIPVAAGELARKEDIDAVIAIGVLIRGATPHFDYIASEVSKGLADLSLELRKPITFGVITADTLEQAIERAGTKHGNKGWEAALSAIEMANLFKSLRGGSGGSGGSGGSGGGDTITLPCNGTGPPPHCSSNITGLILTRQGGYSNDNTVIFRPSGGDWRDIARCNITGTVVSTQLFLNGSLAGNGTVIRSEDWRDNAKSICVQLNTSVEINCTGAGHCNISRAKWNNTLKQIASKLREQYGNKTIIFKPSSGGDPEFVNHSFNCGGEFFYCDSTQLFNSTWFNST

SEQ ID NO: 52 - protein, 360 aa, Artificial Sequence
  recombinant gp120 lumazine synthase fusion protein
MGWSCIILFLVATATGVHSMQIYEGKLTAEGLRFGIVASRFNHALVDRLVEGAIDAIVRHGGREEDITLVRVPGSWEIPVAAGELARKEDIDAVIAIGVLIRGATPHFDYIASEVSKGLADLSLELRKPITFGVITADTLEQAIERAGTKHGNKGWEAALSAIEMANLFKSLRGGSGGSGGSGGSGGGDTITLPCRPAPPPNCTSNITGLILTRQGGYSNDNTVIFRPSGGDWRDIARCNITGTVVSTQLFLNGSLAGNGTVIRSEDWRDNAKSICVQLNTSVEINCTGNGTCNISRAKWNNTLKQIASKLREQYGNKTIIFKPSSGGDPEFVNHSFNCGNVTFYCDSTQLFNSTWFNST

SEQ ID NO: 53 - protein, 360 aa, Artificial Sequence
  recombinant gp120 lumazine synthase fusion protein
MGWSCIILFLVATATGVHSMQIYEGKLTAEGLRFGIVASRFNHALVDRLVEGAIDAIVRHGGREEDITLVRVPGSWEIPVAAGELARKEDIDAVIAIGVLIRGATPHFDYIASEVSKGLADLSLELRKPITFGVITADTLEQAIERAGTKHGNKGWEAALSAIEMANLFKSLRGGSGGSGGSGGSGGGDTITLPCRPAPPPNCTSNITGLILTRQGGYSNDNTVIFRPSGGDWRDIARCNITGTVVSTQLFLNGSLAGNGTVIRSEDWRDNAKSICVQLNTSVEINCTGNGTCNISRAKWNNTLKQIASKLREQYGNKTIIFKPSSGGDPEFVNHSFNCTGEFFYCDSTQLFNSTWFNST

SEQ ID NO: 54 - protein, 360 aa, Artificial Sequence
  recombinant gp120 lumazine synthase fusion protein
MGWSCIILFLVATATGVHSMQIYEGKLTAEGLRFGIVASRFNHALVDRLVEGAIDAIVRHGGREEDITLVRVPGSWEIPVAAGELARKEDIDAVIAIGVLIRGATPHFDYIASEVSKGLADLSLELRKPITFGVITADTLEQAIERAGTKHGNKGWEAALSAIEMANLFKSLRGGSGGSGGSGGSGGGDNITLPCRPAPPPNCTSNITGLILTRQGGYSNDNTVIFRPSGGDWRDIARCNITGNVTSTQLFLNGSLAGNGTVIRSEDWRDNAKSICVQLNTSVEINCTGAGHCNISRAKWNNTLKQIASKLREQYGNKTIIFKPSSGGDPEFVNHSFNCTGEFFYCDSTQLFNSTWFNST

SEQ ID NO: 55 - protein, 360 aa, Artificial Sequence
  recombinant gp120 lumazine synthase fusion protein
MGWSCIILFLVATATGVHSMQIYEGKLTAEGLRFGIVASRFNHALVDRLVEGAIDAIVRHGGREEDITLVRVPGSWEIPVAAGELARKEDIDAVIAIGVLIRGATPHFDYIASEVSKGLADLSLELRKPITFGVITADTLEQAIERAGTKHGNKGWEAALSAIEMANLFKSLRGGSGGSGGSGGSGGGDNITLPCRPAPPPNCTSNITGLILTRQGGYSNDNTVIFRPSGGDWRDIARCQIAGTVVSTQLFLNGSLANGTVVIRSEDWRDNAKSICVQLNTSVEINCTGNGTCNISRAKWNNTLKQIASKLREQYGNKTIIFKPSSGGDPEFVNHSFNCTGEFFYCDSTQLFNSTWFNST

SEQ ID NO: 56 - protein, 361 aa, Artificial Sequence
  recombinant gp120 lumazine synthase fusion protein
MGWSCIILFLVATATGVHSMQIYEGKLTAEGLRFGIVASRFNHALVDRLVEGAIDAIVRHGGREEDITLVRVPGSWEIPVAAGELARKEDIDAVIAIGVLIRGATPHFDYIASEVSKGLADLSLELRKPITFGVITADTLEQAIERAGTKHGNKGWEAALSAIEMANLFKSLRGGSGGSGGSGGSGGGDTITLPCNGTGPPPNCTSNITGLILTRQGGYSNDNTVIFRPSGGDWRDIARCNITGTVVSTQLFLNGSLANGTVVIRSEDWRDNAKSICVQLNTSVEINCTGNGTCNISRAKWNNTLKQIASKLREQYGNKTIIFKPSSGGDPEFVNHSFNCGNVTFYCDSTQLFNSTWFNST

SEQ ID NO: 57 - protein, 360 aa, Artificial Sequence
  recombinant gp120 lumazine synthase fusion protein
MGWSCIILFLVATATGVHSMQIYEGKLTAEGLRFGIVASRFNHALVDRLVEGAIDAIVRHGGREEDITLVRVPGSWEIPVAAGELARKEDIDAVIAIGVLIRGATPHFDYIASEVSKGLADLSLELRKPITFGVITADTLEQAIERAGTKHGNKGWEAALSAIEMANLFKSLRGGSGGSGGSGGSGGGDTITLPCRPAPPPHCSSNITGLILTRQGGYSNDNTVIFRPSGGDWRDIARCQIAGTVVSTQLFLNGSLAGNGTVIRSEDWRDNAKSICVNLTTSVEINCTGNGTCNISRAKWNNTLKQIASKLREQYGNKTIIFKPSSGGDPEFVNHSFNCGNVTFYCDSTQLFNSTWFNST

SEQ ID NO: 58 - protein, 360 aa, Artificial Sequence
  recombinant gp120 lumazine synthase fusion protein
MGWSCIILFLVATATGVHSMQIYEGKLTAEGLRFGIVASRFNHALVDRLVEGAIDAIVRHGGREEDITLVRVPGSWEIPVAAGELARKEDIDAVIAIGVLIRGATPHFDYIASEVSKGLADLSLELRKPITFGVITADTLEQAIERAGTKHGNKGWEAALSAIEMANLFKSLRGGSGGSGGSGGSGGGDTITLPCRPAPPPHCSSNITGLILTRQGGYSNDNTVIFRPSGGDWRDIARCNITGTVVSTQLFLNGSLAGNGTVIRSEDWRDNAKSICVQLNTSVEINCTGNGTCNISRAKWNNTLKQIASKLREQYGNKTIIFKPSSGGDPEFVNHSFNCGNVTFYCDSTQLFNSTWFNST

SEQ ID NO: 59 - protein, 360 aa, Artificial Sequence
  recombinant gp120 lumazine synthase fusion protein
MGWSCIILFLVATATGVHSMQIYEGKLTAEGLRFGIVASRFNHALVDRLVEGAIDAIVRHGGREEDITLVRVPGSWEIPVAAGELARKEDIDAVIAIGVLIRGATPHFDYIASEVSKGLADLSLELRKPITFGVITADTLEQAIERAGTKHGNKGWEAALSAIEMANLFKSLRGGSGGSGGSGGSGGGDTITLPCRPAPPPHCSSNITGLILTRQGGYSNDNTVIFRPSGGDWRDIARCQIAGNVTSTQLFLNGSLAGNGTVIRSEDWRDNAKSICVQLNTSVEINCTGNGTCNISRAKWNNTLKQIASKLREQYGNKTIIFKPSSGGDPEFVNHSFNCGNVTFYCDSTQLFNSTWFNST

SEQ ID NO: 60 - protein, 361 aa, Artificial Sequence
  recombinant gp120 lumazine synthase fusion protein
MGWSCIILFLVATATGVHSMQIYEGKLTAEGLRFGIVASRFNHALVDRLVEGAIDAIVRHGGREEDITLVRVPGSWEIPVAAGELARKEDIDAVIAIGVLIRGATPHFDYIASEVSKGLADLSLELRKPITFGVITADTLEQAIERAGTKHGNKGWEAALSAIEMANLFKSLRGGSGGSGGSGGSGGGDTITLPCNGTGPPPHCSSNITGLILTRQGGYSNDNTVIFRPSGGDWRDIARCNITGTVVSTQLFLNGSLAGNGTVIRSEDWRDNAKSICVQLNTSVEINCTGAGHCNISRAKWNNTLKQIASKLREQYGNKTIIFKPSSGGDPEFVNHSFNCGNVTFYCDSTQLFNSTWFNST

SEQ ID NO: 61 - protein, 361 aa, Artificial Sequence
  recombinant gp120 lumazine synthase fusion protein
MGWSCIILFLVATATGVHSMQIYEGKLTAEGLRFGIVASRFNHALVDRLVEGAIDAIVRHGGREEDITLVRVPGSWEIPVAAGELARKEDIDAVIAIGVLIRGATPHFDYIASEVSKGLADLSLELRKPITFGVITADTLEQAIERAGTKHGNKGWEAALSAIEMANLFKSLRGGSGGSGGSGGSGGGDNITLPCNGTGPPPHCSSNITGLILTRQGGYSNDNTVIFRPSGGDWRDIARCNITGTVVSTQLFLNGSLAGNGTVIRSEDWRDNAKSICVQLNTSVEINCTGAGHCNISRAKWNNTLKQIASKLREQYGNKTIIFKPSSGGDPEFVNHSFNCGNVTFYCDSTQLFNSTWFNST

SEQ ID NO: 62 - protein, 361 aa, Artificial Sequence
  recombinant gp120 lumazine synthase fusion protein
MGWSCIILFLVATATGVHSMQIYEGKLTAEGLRFGIVASRFNHALVDRLVEGAIDAIVRHGGREEDITLVRVPGSWEIPVAAGELARKEDIDAVIAIGVLIRGATPHFDYIASEVSKGLADLSLELRKPITFGVITADTLEQAIERAGTKHGNKGWEAALSAIEMANLFKSLRGGSGGSGGSGGSGGGDNITLPCNGTGPPPHCSSNITGLILTRQGGYSNDNTVIFRPSGGDWRDIARCNITGTVVSTQLFLNGSLAGNGTVIRSEDWRDNAKSICVQLNTSVEINCTGAGHCNISRAKWNNTLKQIASKLREQYGNKTIIFKPSSGGDPEFVNHSFNCGGEFFYCNSTQLFNSTWFNST

SEQ ID NO: 63 - protein, 361 aa, Artificial Sequence
  recombinant gp120 lumazine synthase fusion protein
MGWSCIILFLVATATGVHSMQIYEGKLTAEGLRFGIVASRFNHALVDRLVEGAIDAIVRHGGREEDITLVRVPGSWEIPVAAGELARKEDIDAVIAIGVLIRGATPHFDYIASEVSKGLADLSLELRKPITFGVITADTLEQAIERAGTKHGNKGWEAALSAIEMANLFKSLRGGSGGSGGSGGSGGGDTITLPCNGTGPPPHCSSNITGLILTRQGGYSNDNTVIFRPSGGDWRDIARCNITGTVVSTQLFLNGSLAGNGTVIRSEDWRDNAKSICVQLNTSVEINCTGNGTCNISRAKWNNTLKQIASKLREQYGNKTIIFKPSSGGDPEFVNHSFNCGNVTFYCDSTQLFNSTWFNST

SEQ ID NO: 64 - protein, 361 aa, Artificial Sequence
  recombinant gp120 lumazine synthase fusion protein
MGWSCIILFLVATATGVHSMQIYEGKLTAEGLRFGIVASRFNHALVDRLVEGAIDAIVRHGGREEDITLVRVPGSWEIPVAAGELARKEDIDAVIAIGVLIRGATPHFDYIASEVSKGLADLSLELRKPITFGVITADTLEQAIERAGTKHGNKGWEAALSAIEMANLFKSLRGGSGGSGGSGGSGGGDTITLPCNGTGPPPHCSSNITGLILTRQGGYSNDNTVIFRPSGGDWRDIARCNITGTVVSTQLFLNGSLAGNGTVIRSEDWRDNAKSICVQLNTSVEINCTGAGHCNISRAKWNNTLKQIASKLREQYGNKTIIFKPSSGGDPEFVNHSFNCGNVTFYCNSTQLFNSTWFNST

SEQ ID NO: 65 - protein, 361 aa, Artificial Sequence
  recombinant gp120 lumazine synthase fusion protein
MGWSCIILFLVATATGVHSMQIYEGKLTAEGLRFGIVASRFNHALVDRLVEGAIDAIVRHGGREEDITLVRVPGSWEIPVAAGELARKEDIDAVIAIGVLIRGATPHFDYIASEVSKGLADLSLELRKPITFGVITADTLEQAIERAGTKHGNKGWEAALSAIEMANLFKSLRGGSGGSGGSGGSGGGDTITLPCNGTGPPPHCSSNITGLILTRQGGYSNDNTVIFRPSGGDWRDIARCNITGTVVSTQLFLNGSLAGNGTVIRSEDWRDNAKSICVQLNTSVEINCTGNGTCNISRAKWNNTLKQIASKLREQYGNKTIIFKPSSGGDPEFVNHSFNCGGEFFYCNSTQLFNSTWFNST

SEQ ID NO: 66 - protein, 856 aa, Human immunodeficiency virus type 1
MRVKEKYQHLWRWGWRWGTMLLGMLMICSATEKLWVTVYYGVPVWKEATTTLFCASDAKAYDTEVHNVWATHACVPTDPNPQEVVLVNVTENFNMWKNDMVEQMHEDIISLWDQSLKPCVKLTPLCVSLKCTDLKNDTNTNSSSGRMIMEKGEIKNCSFNISTSIRGKVQKEYAFFYKLDIIPIDNDTTSYKLTSCNTSVITQACPKVSFEPIPIHYCAPAGFAILKCNNKTFNGTGPCTNVSTVQCTHGIRPVVSTQLLLNGSLAEEEVVIRSVNFTDNAKTIIVQLNTSVEINCTRPNNNTRKRIRIQRGPGRAFVTIGKIGNMRQAHCNISRAKWNNTLKQIASKLREQFGNNKTIIFKQSSGGDPEIVTHSFNCGGEFFYCNSTQLFNSTWFNSTWSTEGSNNTEGSDTITLPCRIKQIINMWQKVGKAMYAPPISGQIRCSSNITGLLLTRDGGNSNNESEIFRPGGGDMRDNWRSELYKYKVVKIEPLGVAPTKAKRRVVQREKRAVGIGALFLGFLGAAGSTMGAASMTLTVQARQLLSGIVQQQNNLLRAIEAQQHLLQLTVWGIKQLQARILAVERYLKDQQLLGIWGCSGKLICTTAVPWNASWSNKSLEQIWNHTTWMEWDREINNYTSLIHSLIEESQNQQEKNEQELLELDKWASLWNWFNITNWLWYIKLFIMIVGGLVGLRIVFAVLSIVNRVRQGYSPLSFQTHLPTPRGPDRPEGIEEEGGERDRDRSIRLVNGSLALIWDDLRSLCLFSYHRLRDLLLIVTRIVELLGRRGWEALKYWWNLLQYWSQELKNSAVSLLNATAIAVAEGTDRVIEVVQGACRAIRHIPRRIRQGLERILL

SEQ ID NO: 67 - protein, 154 aa, Artificial Sequence
  recombinant lumazine synthase subunit
MQIYEGKLTAEGLRFGIVASRFNHALVDRLVEGAIDAIVRHGGREEDITLVRVPGSWEIPVAAGELARKEDIDAVIAIGVLIRGATPHFDYIASEVSKGLADLSLELRKPITFGVITADTLEQAIEAAGTKHGNKGWEAALSAIEMANLFKSLR

SEQ ID NO: 68 - protein, 154 aa, Artificial Sequence
  recombinant lumazine synthase subunit
MQIYEGKLTAEGLRFGIVASRFNHALVDRLVEGAIDAIVRHGGREEDITLVRVPGSWEIPVAAGELARKEDIDAVIAIGVLIRGATPSFDYIASEVSKGLADLSLELRKPITFGVITADTLEQAIEAAGTKHGNKGWEAALSAIEMANLFKSLR

SEQ ID NO: 69 - protein, 154 aa, Artificial Sequence
  recombinant lumazine synthase subunit
MQIYEGKLTAEGLRFGIVASRANHALVDRLVEGAIDAIVRHGGREEDITLVRVPGSWEIPVAAGELARKEDIDAVIAIGVLIRGATPSFDYIASEVSKGLADLSLELRKPITFGVITADTLEQAIEAAGTKHGNKGWEAALSAIEMANLFKSLR

SEQ ID NO: 70 - protein, 173 aa, Artificial Sequence
  recombinant ferritin subunit
ESQVRQQFSKDIEKLLNEQVNKEMQSSNLYMSMSSWCYTHSLDGAGLFLFDHAAEEYEHAKKLIIFLNENNVPVQLTSISAPEHKFEGLTQIFQKAYEHEQHISESINNIVDHAIKSKDHATFNFLQWYVAEQHEEEVLFKDILDKIELIGNENHGLYLADQYVKGIAKSRKS

SEQ ID NO: 71 - protein, 265 aa, Artificial Sequence [sequence omitted]

SEQ ID NO: 72 - protein, 265 aa, Artificial Sequence [sequence omitted]

SEQ ID NO: 73 - protein, 27 aa, Artificial Sequence
  Transmembrane domain
KIFIMIVGGLIGLRIVFAVLSVIHRVR

SEQ ID NO: 74 - protein, 23 aa, Artificial Sequence
  Transmembrane domain
ILAIYSTVASSLVLLVSLGAISF

SEQ ID NO: 75 - protein, 29 aa, Artificial Sequence
  Transmembrane domain
IITIGSICMVVGIISLILQIGNIISIWVS

SEQ ID NO: 76 - protein, 360 aa, Artificial Sequence
  recombinant gp120 lumazine synthase fusion protein
MGWSCIILFLVATATGVHSMQIYEGKLTAEGLRFGIVASRFNHALVDRLVEGAIDAIVRHGGREEDITLVRVPGSWEIPVAAGELARKEDIDAVIAIGVLIRGATPHFDYIASEVSKGLADLSLELRKPITFGVITADTLEQAIERAGTKHGNKGWEAALSAIEMANLFKSLRGGSGGSGGSGGSGGGDTITLPCRPAPPPHCSSNITGLILTRQGGYSNDNTVIFRPSGGDWRDIARCNITGTVVSTQLFLNGSLAGNGTVIRSENFTDNAKSICVQLNTSVEINCTGNGTCNISRAKWNNTLKQIASKLREQYGNKTIIFKPSSGGDPEFVNHSFNCGNVTFYCDSTQLFNSTWFNST

SEQ ID NO: 77 - protein, 172 aa, Artificial Sequence
  recombinant gp120 protein
DTITLPCRPAPPPHCSSNITGLILTRQGGYSNDNTVIFRPSGGDWRDIARCQIAGTVVSTQLFLNGSLAGNGTVIRSEDWRDNAKSICVQLNTSVEINCTGAGHCNISRAKWNNTLKQIASKLREQYGNKTIIFKPSSGGDPEFVNHSFNCGGEFFYCDSTQLFNSTWFNST

SEQ ID NO: 78 - protein, 5 aa, Artificial Sequence
  recombinant gp120 protein fragment
QQYEF

SEQ ID NO: 79 - protein, 172 aa, Artificial Sequence
  recombinant gp120 protein
DTITLPCRPAPPPHCSSNITGLILTRQGGYSNDNTVIFRPSGGDWRDIARCQIAGNVTSTQLFLNGSLAGNGTVIRSEDWRDNAKSICVQLNTSVEINCTGAGHCNISRAKWNNTLKQIASKLREQYGNKTIIFKPSSGGDPEFVNHSFNCGNVTFYCDSTQLFNSTWFNST

SEQ ID NO: 80 - protein, 172 aa, Artificial Sequence
  recombinant gp120 protein
DTITLPCRPAPPPHCSSNITGLILTRQGGYSNDNTVIFRPSGGDWRDIARCQIAGNVTSTQLFLNGSLAGGEVNGTSEDWRDNAKSICVQLNTSVEINCTGAGHCNISRAKWNNTLKQIASKLREQYGNKTIIFKPSSGGDPEFVNHSFNCGNVTFYCDSTQLFNSTWFNST

SEQ ID NO: 81 - protein, 173 aa, Artificial Sequence
  recombinant gp120 protein
DTITLPCNGTGPPPHCSSNITGLILTRQGGYSNDNTVIFRPSGGDWRDIARCQIAGNVTSTQLFLNGSLANGTVNGTSEDWRDNAKSICVQLNTSVEINCTGAGHCNISRAKWNNTLKQIASKLREQYGNKTIIFKPSSGGDPEFVNHSFNCGNVTFYCDSTQLFNSTWFNST

SEQ ID NO: 82 - protein, 172 aa, Artificial Sequence
  recombinant gp120 protein
DTITLPCRPAPPPNCTSNITGLILTRQGGYSNDNTVIFRPSGGDWRDIARCQIAGTVVSTQLFLNGSLAGNGTVIRSEDWRDNAKSICVQLNTSVEINCTGNGTCNISRAKWNNTLKQIASKLREQYGNKTIIFKPSSGGDPEFVNHSFNCGNVTFYCDSTQLFNSTWFNST

SEQ ID NO: 83 - protein, 360 aa, Artificial Sequence
  recombinant gp120 lumazine synthase fusion protein
MGWSCIILFLVATATGVHSMQIYEGKLTAEGLRFGIVASRFNHALVDRLVEGAIDAIVRHGGREEDITLVRVPGSWEIPVAAGELARKEDIDAVIAIGVLIRGATPHFDYIASEVSKGLADLSLELRKPITFGVITADTLEQAIERAGTKHGNKGWEAALSAIEMANLFKSLRGGSGGSGGSGGSGGGDTITLPCRPAPPPHCSSNITGLILTRQGGYSNDNTVIFRPSGGDWRDIARCQIAGNVTSTQLFLNGSLAGNGTVIRSEDWRDNAKSICVQLNTSVEINCTGAGHCNISRAKWNNTLKQIASKLREQYGNKTIIFKPSSGGDPEFVNHSFNCGNVTFYCDSTQLFNSTWFNST

SEQ ID NO: 84 - protein, 360 aa, Artificial Sequence
  recombinant gp120 lumazine synthase fusion protein
MGWSCIILFLVATATGVHSMQIYEGKLTAEGLRFGIVASRFNHALVDRLVEGAIDAIVRHGGREEDITLVRVPGSWEIPVAAGELARKEDIDAVIAIGVLIRGATPHFDYIASEVSKGLADLSLELRKPITFGVITADTLEQAIERAGTKHGNKGWEAALSAIEMANLFKSLRGGSGGSGGSGGSGGGDTITLPCRPAPPPHCSSNITGLILTRQGGYSNDNTVIFRPSGGDWRDIARCQIAGNVTSTQLFLNGSLAGGEVNGTSEDWRDNAKSICVQLNTSVEINCTGAGHCNISRAKWNNTLKQIASKLREQYGNKTIIFKPSSGGDPEFVNHSFNCGNVTFYCDSTQLFNSTWFNST

SEQ ID NO: 85 - protein, 361 aa, Artificial Sequence
  recombinant gp120 lumazine synthase fusion protein
MGWSCIILFLVATATGVHSMQIYEGKLTAEGLRFGIVASRFNHALVDRLVEGAIDAIVRHGGREEDITLVRVPGSWEIPVAAGELARKEDIDAVIAIGVLIRGATPHFDYIASEVSKGLADLSLELRKPITFGVITADTLEQAIERAGTKHGNKGWEAALSAIEMANLFKSLRGGSGGSGGSGGSGGGDTITLPCNGTGPPPHCSSNITGLILTRQGGYSNDNTVIFRPSGGDWRDIARCQIAGNVTSTQLFLNGSLANGTVNGTSEDWRDNAKSICVQLNTSVEINCTGAGHCNISRAKWNNTLKQIASKLREQYGNKTIIFKPSSGGDPEFVNHSFNCGNVTFYCDSTQLFNSTWFNST

SEQ ID NO: 86 - protein, 360 aa, Artificial Sequence
  recombinant gp120 lumazine synthase fusion protein
MGWSCIILFLVATATGVHSMQIYEGKLTAEGLRFGIVASRFNHALVDRLVEGAIDAIVRHGGREEDITLVRVPGSWEIPVAAGELARKEDIDAVIAIGVLIRGATPHFDYIASEVSKGLADLSLELRKPITFGVITADTLEQAIERAGTKHGNKGWEAALSAIEMANLFKSLRGGSGGSGGSGGSGGGDTITLPCRPAPPPNCTSNITGLILTRQGGYSNDNTVIFRPSGGDWRDIARCQIAGTVVSTQLFLNGSLAGNGTVIRSEDWRDNAKSICVQLNTSVEINCTGNGTCNISRAKWNNTLKQIASKLREQYGNKTIIFKPSSGGDPEFVNHSFNCGNVTFYCDSTQLFNSTWFNST

SEQ ID NO: 87 - DNA, 1104 bp, Artificial Sequence
  recombinant gp120 lumazine synthase fusion protein
atgcccatgggcagcctgcagcccctggccaccctgtacctgctgggcatgctggtggctagcgtgctggccatgcagatctacgaaggcaagctgaccgccgaggggctgagattcggaattgtggcaagcaggtttaaccacgcactggtggaccgactggtcgaaggagctatcgatgcaattgtgcggcatggcgggagagaggaagacatcacactggtgagagtcccaggcagctgggagattccagtggcagctggagaactggcacggaaagaggacatcgatgccgtgatcgctattggcgtcctgattagaggggctactccccacttcgactatatcgcatcagaagtgagcaagggcctggccgatctgtctctggagctgcgaaaacctatcacttttggggtcattactgccgataccctggaacaggcaatcgagcgcgccggcaccaagcatggaaacaaaggctgggaagcagccctgtccgctattgagatggcaaatctgttcaagtctctgaggggaggctccggaggctccggcggctctggcggcagcggcggaggcgacaccatcacactgccatgcaacggaaccggaccacctccacactgtagctccaatatcaccggactgatcctgacaaggcagggaggctactccaacgataatacagtgatcttcagaccatctggcggcgactggagggatatcgcaagatgcaatatcaccggcacagtggtgagcacccagctgtttctgaacggctccctggccggcaatggcacagtgatcaggtccgaggactggcgcgataacgccaagtctatctgcgtgcagctgaacaccagcgtggagatcaattgcacaggcgccggccactgtaatatctctagggccaagtggaacaataccctgaagcagatcgccagcaagctgagagagcagtacggcaacaagacaatcatcttcaagccctctagcggcggcgaccctgagttcgtgaaccacagctttaattgcggcggcgagttcttttattgtgattccacccagctgttcaactccacctggtttaattctacatgatga

SEQ ID NO: 88 - DNA, 1101 bp, Artificial Sequence
  recombinant gp120 lumazine synthase fusion protein
atgcccatgggcagcctgcagcccctggccaccctgtacctgctgggcatgctggtggctagcgtgctggccatgcagatctacgaaggcaagctgaccgccgaggggctgagattcggaattgtggcaagcaggtttaaccacgcactggtggaccgactggtcgaaggagctatcgatgcaattgtgcggcatggcgggagagaggaagacatcacactggtgagagtcccaggcagctgggagattccagtggcagctggagaactggcacggaaagaggacatcgatgccgtgatcgctattggcgtcctgattagaggggctactccccacttcgactatatcgcatcagaagtgagcaagggcctggccgatctgtctctggagctgcgaaaacctatcacttttggggtcattactgccgataccctggaacaggcaatcgagcgcgccggcaccaagcatggaaacaaaggctgggaagcagccctgtccgctattgagatggcaaatctgttcaagtctctgaggggaggctccggaggctctggcggcagcggcggctccggcggaggcgacaccatcacactgccatgcaggcctgcaccacctccaaactgtacctctaatatcacaggactgatcctgaccaggcagggaggatactctaacgataatacagtgatcttcagacctagcggcggcgactggagggatatcgcaagatgcaatatcaccggcacagtggtgtccacccagctgtttctgaatggctctctggccggcaacggcacagtgatcaggagcgaggactggcgcgataatgccaagagcatctgcgtgcagctgaacacctccgtggagatcaactgcaccggcaatggcacatgtaacatcagcagggccaagtggaacaataccctgaagcagatcgcctccaagctgcgcgagcagtacggcaataagacaatcatcttcaagccaagctccggcggcgaccccgagttcgtgaaccactcctttaactgcggcaatgtgaccttttattgtgattctacacagctgttcaattctacctggtttaacagcacatgatga

SEQ ID NO: 89 - DNA, 1104 bp, Artificial Sequence
  recombinant gp120 lumazine synthase fusion protein
atgcccatgggcagcctgcagcccctggccaccctgtacctgctgggcatgctggtggctagcgtgctggccatgcagatctacgaaggcaagctgaccgccgaggggctgagattcggaattgtggcaagcaggtttaaccacgcactggtggaccgactggtcgaaggagctatcgatgcaattgtgcggcatggcgggagagaggaagacatcacactggtgagagtcccaggcagctgggagattccagtggcagctggagaactggcacggaaagaggacatcgatgccgtgatcgctattggcgtcctgattagaggggctactccccacttcgactatatcgcatcagaagtgagcaagggcctggccgatctgtctctggagctgcgaaaacctatcacttttggggtcattactgccgataccctggaacaggcaatcgagcgcgccggcaccaagcatggaaacaaaggctgggaagcagccctgtccgctattgagatggcaaatctgttcaagtctctgaggggaggctccggaggctccggcggctctggcggcagcggcggaggcgacaccatcacactgccatgcaacggaaccggaccacctccacactgtagctccaatatcaccggactgatcctgacaaggcagggaggctactccaacgataatacagtgatcttcagaccatctggcggcgactggagggatatcgcaagatgcaatatcaccggcacagtggtgagcacccagctgtttctgaacggctccctggccggcaatggcacagtgatcaggtccgaggactggcgcgataacgccaagtctatctgcgtgcagctgaacaccagcgtggagatcaattgcacaggcgccggccactgtaatatctctagggccaagtggaacaataccctgaagcagatcgccagcaagctgagagagcagtacggcaacaagacaatcatcttcaagccctctagcggcggcgaccctgagttcgtgaaccacagctttaattgcggcaacgtgaccttttattgtgattccacccagctgttcaactccacctggtttaattctacatgatga

SEQ ID NO: 90 - DNA, 525 bp, Artificial Sequence
  recombinant gp120 protein
gacaccatcacactgccatgcaacggaaccggaccacctccacactgtagctccaatatcaccggactgatcctgacaaggcagggaggctactccaacgataatacagtgatcttcagaccatctggcggcgactggagggatatcgcaagatgcaatatcaccggcacagtggtgagcacccagctgtttctgaacggctccctggccggcaatggcacagtgatcaggtccgaggactggcgcgataacgccaagtctatctgcgtgcagctgaacaccagcgtggagatcaattgcacaggcgccggccactgtaatatctctagggccaagtggaacaataccctgaagcagatcgccagcaagctgagagagcagtacggcaacaagacaatcatcttcaagccctctagcggcggcgaccctgagttcgtgaaccacagctttaattgcggcggcgagttcttttattgtgattccacccagctgttcaactccacctggtttaattctacatgatga

SEQ ID NO: 91 - DNA, 522 bp, Artificial Sequence
  recombinant gp120 protein
gacaccatcacactgccatgcaggcctgcaccacctccaaactgtacctctaatatcacaggactgatcctgaccaggcagggaggatactctaacgataatacagtgatcttcagacctagcggcggcgactggagggatatcgcaagatgcaatatcaccggcacagtggtgtccacccagctgtttctgaatggctctctggccggcaacggcacagtgatcaggagcgaggactggcgcgataatgccaagagcatctgcgtgcagctgaacacctccgtggagatcaactgcaccggcaatggcacatgtaacatcagcagggccaagtggaacaataccctgaagcagatcgcctccaagctgcgcgagcagtacggcaataagacaatcatcttcaagccaagctccggcggcgaccccgagttcgtgaaccactcctttaactgcggcaatgtgaccttttattgtgattctacacagctgttcaattctacctggtttaacagcacatgatga

SEQ ID NO: 92 - DNA, 525 bp, Artificial Sequence
  recombinant gp120 protein
gacaccatcacactgccatgcaacggaaccggaccacctccacactgtagctccaatatcaccggactgatcctgacaaggcagggaggctactccaacgataatacagtgatcttcagaccatctggcggcgactggagggatatcgcaagatgcaatatcaccggcacagtggtgagcacccagctgtttctgaacggctccctggccggcaatggcacagtgatcaggtccgaggactggcgcgataacgccaagtctatctgcgtgcagctgaacaccagcgtggagatcaattgcacaggcgccggccactgtaatatctctagggccaagtggaacaataccctgaagcagatcgccagcaagctgagagagcagtacggcaacaagacaatcatcttcaagccctctagcggcggcgaccctgagttcgtgaaccacagctttaattgcggcaacgtgaccttttattgtgattccacccagctgttcaactccacctggtttaattctacatgatga

SEQ ID NO: 93 - protein, 178 aa, Artificial sequence
  lumazine synthase nanoparticle sequence
MPMGSLQPLATLYLLGMLVASVLAMQIYEGKLTAEGLRFGIVASRFNHALVDRLVEGAIDAIVRHGGREEDITLVRVPGSWEIPVAAGELARKEDIDAVIAIGVLIRGATPHFDYIASEVSKGLADLSLELRKPITFGVITADTLEQAIERAGTKHGNKGWEAALSAIEMANLFKSLR

SEQ ID NO: 94 - protein, 366 aa, Artificial sequence
  recombinant gp120 lumazine synthase fusion protein
MPMGSLQPLATLYLLGMLVASVLAMQIYEGKLTAEGLRFGIVASRFNHALVDRLVEGAIDAIVRHGGREEDITLVRVPGSWEIPVAAGELARKEDIDAVIAIGVLIRGATPHFDYIASEVSKGLADLSLELRKPITFGVITADTLEQAIERAGTKHGNKGWEAALSAIEMANLFKSLRGGSGGSGGSGGSGGGDTITLPCNGTGPPPHCSSNITGLILTRQGGYSNDNTVIFRPSGGDWRDIARCNITGTVVSTQLFLNGSLAGNGTVIRSEDWRDNAKSICVQLNTSVEINCTGAGHCNISRAKWNNTLKQIASKLREQYGNKTIIFKPSSGGDPEFVNHSFNCGGEFFYCDSTQLFNSTWFNST

SEQ ID NO: 95 - protein, 365 aa, Artificial sequence
  recombinant gp120 lumazine synthase fusion protein
MPMGSLQPLATLYLLGMLVASVLAMQIYEGKLTAEGLRFGIVASRFNHALVDRLVEGAIDAIVRHGGREEDITLVRVPGSWEIPVAAGELARKEDIDAVIAIGVLIRGATPHFDYIASEVSKGLADLSLELRKPITFGVITADTLEQAIERAGTKHGNKGWEAALSAIEMANLFKSLRGGSGGSGGSGGSGGGDTITLPCRPAPPPNCTSNITGLILTRQGGYSNDNTVIFRPSGGDWRDIARCNITGTVVSTQLFLNGSLAGNGTVIRSEDWRDNAKSICVQLNTSVEINCTGNGTCNISRAKWNNTLKQIASKLREQYGNKTIIFKPSSGGDPEFVNHSFNCGNVTFYCDSTQLFNSTWFNST

SEQ ID NO: 96 - protein, 365 aa, Artificial sequence
  recombinant gp120 lumazine synthase fusion protein
MPMGSLQPLATLYLLGMLVASVLAMQIYEGKLTAEGLRFGIVASRFNHALVDRLVEGAIDAIVRHGGREEDITLVRVPGSWEIPVAAGELARKEDIDAVIAIGVLIRGATPHFDYIASEVSKGLADLSLELRKPITFGVITADTLEQAIERAGTKHGNKGWEAALSAIEMANLFKSLRGGSGGSGGSGGSGGGDTITLPCRPAPPPNCTSNITGLILTRQGGYSNDNTVIFRPSGGDWRDIARCNITGTVVSTQLFLNGSLAGNGTVIRSEDWRDNAKSICVQLNTSVEINCTGNGTCNISRAKWNNTLKQIASKLREQYGNKTIIFKPSSGGDPEFVNHSFNCTGEFFYCDSTQLFNSTWFNST

SEQ ID NO: 97 - protein, 365 aa, Artificial sequence
  recombinant gp120 lumazine synthase fusion protein
MPMGSLQPLATLYLLGMLVASVLAMQIYEGKLTAEGLRFGIVASRFNHALVDRLVEGAIDAIVRHGGREEDITLVRVPGSWEIPVAAGELARKEDIDAVIAIGVLIRGATPHFDYIASEVSKGLADLSLELRKPITFGVITADTLEQAIERAGTKHGNKGWEAALSAIEMANLFKSLRGGSGGSGGSGGSGGGDNITLPCRPAPPPNCTSNITGLILTRQGGYSNDNTVIFRPSGGDWRDIARCNITGNVTSTQLFLNGSLAGNGTVIRSEDWRDNAKSICVQLNTSVEINCTGAGHCNISRAKWNNTLKQIASKLREQYGNKTIIFKPSSGGDPEFVNHSFNCTGEFFYCDSTQLFNSTWFNST

SEQ ID NO: 98 - protein, 365 aa, Artificial sequence
  recombinant gp120 lumazine synthase fusion protein
MPMGSLQPLATLYLLGMLVASVLAMQIYEGKLTAEGLRFGIVASRFNHALVDRLVEGAIDAIVRHGGREEDITLVRVPGSWEIPVAAGELARKEDIDAVIAIGVLIRGATPHFDYIASEVSKGLADLSLELRKPITFGVITADTLEQAIERAGTKHGNKGWEAALSAIEMANLFKSLRGGSGGSGGSGGSGGGDNITLPCRPAPPPNCTSNITGLILTRQGGYSNDNTVIFRPSGGDWRDIARCQIAGTVVSTQLFLNGSLANGTVVIRSEDWRDNAKSICVQLNTSVEINCTGNGTCNISRAKWNNTLKQIASKLREQYGNKTIIFKPSSGGDPEFVNHSFNCTGEFFYCDSTQLFNSTWFNST

SEQ ID NO: 99 - protein, 366 aa, Artificial sequence
  recombinant gp120 lumazine synthase fusion protein
MPMGSLQPLATLYLLGMLVASVLAMQIYEGKLTAEGLRFGIVASRFNHALVDRLVEGAIDAIVRHGGREEDITLVRVPGSWEIPVAAGELARKEDIDAVIAIGVLIRGATPHFDYIASEVSKGLADLSLELRKPITFGVITADTLEQAIERAGTKHGNKGWEAALSAIEMANLFKSLRGGSGGSGGSGGSGGGDTITLPCNGTGPPPNCTSNITGLILTRQGGYSNDNTVIFRPSGGDWRDIARCNITGTVVSTQLFLNGSLANGTVVIRSEDWRDNAKSICVQLNTSVEINCTGNGTCNISRAKWNNTLKQIASKLREQYGNKTIIFKPSSGGDPEFVNHSFNCGNVTFYCDSTQLFNSTWFNST

SEQ ID NO: 100 - protein, 365 aa, Artificial sequence
  recombinant gp120 lumazine synthase fusion protein
MPMGSLQPLATLYLLGMLVASVLAMQIYEGKLTAEGLRFGIVASRFNHALVDRLVEGAIDAIVRHGGREEDITLVRVPGSWEIPVAAGELARKEDIDAVIAIGVLIRGATPHFDYIASEVSKGLADLSLELRKPITFGVITADTLEQAIERAGTKHGNKGWEAALSAIEMANLFKSLRGGSGGSGGSGGSGGGDTITLPCRPAPPPHCSSNITGLILTRQGGYSNDNTVIFRPSGGDWRDIARCQIAGTVVSTQLFLNGSLAGNGTVIRSEDWRDNAKSICVNLTTSVEINCTGNGTCNISRAKWNNTLKQIASKLREQYGNKTIIFKPSSGGDPEFVNHSFNCGNVTFYCDSTQLFNSTWFNST

SEQ ID NO: 101 - protein, 365 aa, Artificial sequence
  recombinant gp120 lumazine synthase fusion protein
MPMGSLQPLATLYLLGMLVASVLAMQIYEGKLTAEGLRFGIVASRFNHALVDRLVEGAIDAIVRHGGREEDITLVRVPGSWEIPVAAGELARKEDIDAVIAIGVLIRGATPHFDYIASEVSKGLADLSLELRKPITFGVITADTLEQAIERAGTKHGNKGWEAALSAIEMANLFKSLRGGSGGSGGSGGSGGGDTITLPCRPAPPPHCSSNITGLILTRQGGYSNDNTVIFRPSGGDWRDIARCNITGTVVSTQLFLNGSLAGNGTVIRSEDWRDNAKSICVQLNTSVEINCTGNGTCNISRAKWNNTLKQIASKLREQYGNKTIIFKPSSGGDPEFVNHSFNCGNVTFYCDSTQLFNSTWFNST

SEQ ID NO: 102 - protein, 365 aa, Artificial sequence
  recombinant gp120 lumazine synthase fusion protein
MPMGSLQPLATLYLLGMLVASVLAMQIYEGKLTAEGLRFGIVASRFNHALVDRLVEGAIDAIVRHGGREEDITLVRVPGSWEIPVAAGELARKEDIDAVIAIGVLIRGATPHFDYIASEVSKGLADLSLELRKPITFGVITADTLEQAIERAGTKHGNKGWEAALSAIEMANLFKSLRGGSGGSGGSGGSGGGDTITLPCRPAPPPHCSSNITGLILTRQGGYSNDNTVIFRPSGGDWRDIARCQIAGNVTSTQLFLNGSLAGNGTVIRSEDWRDNAKSICVQLNTSVEINCTGNGTCNISRAKWNNTLKQIASKLREQYGNKTIIFKPSSGGDPEFVNHSFNCGNVTFYCDSTQLFNSTWFNST

SEQ ID NO: 103 - protein, 366 aa, Artificial sequence
  recombinant gp120 lumazine synthase fusion protein
MPMGSLQPLATLYLLGMLVASVLAMQIYEGKLTAEGLRFGIVASRFNHALVDRLVEGAIDAIVRHGGREEDITLVRVPGSWEIPVAAGELARKEDIDAVIAIGVLIRGATPHFDYIASEVSKGLADLSLELRKPITFGVITADTLEQAIERAGTKHGNKGWEAALSAIEMANLFKSLRGGSGGSGGSGGSGGGDTITLPCNGTGPPPHCSSNITGLILTRQGGYSNDNTVIFRPSGGDWRDIARCNITGTVVSTQLFLNGSLAGNGTVIRSEDWRDNAKSICVQLNTSVEINCTGAGHCNISRAKWNNTLKQIASKLREQYGNKTIIFKPSSGGDPEFVNHSFNCGNVTFYCDSTQLFNSTWFNST

SEQ ID NO: 104 - protein, 366 aa, Artificial sequence
  recombinant gp120 lumazine synthase fusion protein
MPMGSLQPLATLYLLGMLVASVLAMQIYEGKLTAEGLRFGIVASRFNHALVDRLVEGAIDAIVRHGGREEDITLVRVPGSWEIPVAAGELARKEDIDAVIAIGVLIRGATPHFDYIASEVSKGLADLSLELRKPITFGVITADTLEQAIERAGTKHGNKGWEAALSAIEMANLFKSLRGGSGGSGGSGGSGGGDNITLPCNGTGPPPHCSSNITGLILTRQGGYSNDNTVIFRPSGGDWRDIARCNITGTVVSTQLFLNGSLAGNGTVIRSEDWRDNAKSICVQLNTSVEINCTGAGHCNISRAKWNNTLKQIASKLREQYGNKTIIFKPSSGGDPEFVNHSFNCGNVTFYCDSTQLFNSTWFNST

SEQ ID NO: 105 - protein, 366 aa, Artificial sequence
  recombinant gp120 lumazine synthase fusion protein
MPMGSLQPLATLYLLGMLVASVLAMQIYEGKLTAEGLRFGIVASRFNHALVDRLVEGAIDAIVRHGGREEDITLVRVPGSWEIPVAAGELARKEDIDAVIAIGVLIRGATPHFDYIASEVSKGLADLSLELRKPITFGVITADTLEQAIERAGTKHGNKGWEAALSAIEMANLFKSLRGGSGGSGGSGGSGGGDNITLPCNGTGPPPHCSSNITGLILTRQGGYSNDNTVIFRPSGGDWRDIARCNITGTVVSTQLFLNGSLAGNGTVIRSEDWRDNAKSICVQLNTSVEINCTGAGHCNISRAKWNNTLKQIASKLREQYGNKTIIFKPSSGGDPEFVNHSFNCGGEFFYCNSTQLFNSTWFNST

SEQ ID NO: 106 - protein, 366 aa, Artificial sequence
  recombinant gp120 lumazine synthase fusion protein
MPMGSLQPLATLYLLGMLVASVLAMQIYEGKLTAEGLRFGIVASRFNHALVDRLVEGAIDAIVRHGGREEDITLVRVPGSWEIPVAAGELARKEDIDAVIAIGVLIRGATPHFDYIASEVSKGLADLSLELRKPITFGVITADTLEQAIERAGTKHGNKGWEAALSAIEMANLFKSLRGGSGGSGGSGGSGGGDTITLPCNGTGPPPHCSSNITGLILTRQGGYSNDNTVIFRPSGGDWRDIARCNITGTVVSTQLFLNGSLAGNGTVIRSEDWRDNAKSICVQLNTSVEINCTGNGTCNISRAKWNNTLKQIASKLREQYGNKTIIFKPSSGGDPEFVNHSFNCGNVTFYCDSTQLFNSTWFNST

SEQ ID NO: 107 - protein, 366 aa, Artificial sequence
  recombinant gp120 lumazine synthase fusion protein
MPMGSLQPLATLYLLGMLVASVLAMQIYEGKLTAEGLRFGIVASRFNHALVDRLVEGAIDAIVRHGGREEDITLVRVPGSWEIPVAAGELARKEDIDAVIAIGVLIRGATPHFDYIASEVSKGLADLSLELRKPITFGVITADTLEQAIERAGTKHGNKGWEAALSAIEMANLFKSLRGGSGGSGGSGGSGGGDTITLPCNGTGPPPHCSSNITGLILTRQGGYSNDNTVIFRPSGGDWRDIARCNITGTVVSTQLFLNGSLAGNGTVIRSEDWRDNAKSICVQLNTSVEINCTGAGHCNISRAKWNNTLKQIASKLREQYGNKTIIFKPSSGGDPEFVNHSFNCGNVTFYCNSTQLFNSTWFNST

SEQ ID NO: 108 - protein, 366 aa, Artificial sequence
  recombinant gp120 lumazine synthase fusion protein
MPMGSLQPLATLYLLGMLVASVLAMQIYEGKLTAEGLRFGIVASRFNHALVDRLVEGAIDAIVRHGGREEDITLVRVPGSWEIPVAAGELARKEDIDAVIAIGVLIRGATPHFDYIASEVSKGLADLSLELRKPITFGVITADTLEQAIERAGTKHGNKGWEAALSAIEMANLFKSLRGGSGGSGGSGGSGGGDTITLPCNGTGPPPHCSSNITGLILTRQGGYSNDNTVIFRPSGGDWRDIARCNITGTVVSTQLFLNGSLAGNGTVIRSEDWRDNAKSICVQLNTSVEINCTGNGTCNISRAKWNNTLKQIASKLREQYGNKTIIFKPSSGGDPEFVNHSFNCGGEFFYCNSTQLFNSTWFNST

SEQ ID NO: 109 - protein, 365 aa, Artificial sequence
  recombinant gp120 lumazine synthase fusion protein
MPMGSLQPLATLYLLGMLVASVLAMQIYEGKLTAEGLRFGIVASRFNHALVDRLVEGAIDAIVRHGGREEDITLVRVPGSWEIPVAAGELARKEDIDAVIAIGVLIRGATPHFDYIASEVSKGLADLSLELRKPITFGVITADTLEQAIERAGTKHGNKGWEAALSAIEMANLFKSLRGGSGGSGGSGGSGGGDTITLPCRPAPPPHCSSNITGLILTRQGGYSNDNTVIFRPSGGDWRDIARCNITGTVVSTQLFLNGSLAGNGTVIRSENFTDNAKSICVQLNTSVEINCTGNGTCNISRAKWNNTLKQIASKLREQYGNKTIIFKPSSGGDPEFVNHSFNCGNVTFYCDSTQLFNSTWFNST

SEQ ID NO: 110 - protein, 365 aa, Artificial sequence
  recombinant gp120 lumazine synthase fusion protein
MPMGSLQPLATLYLLGMLVASVLAMQIYEGKLTAEGLRFGIVASRFNHALVDRLVEGAIDAIVRHGGREEDITLVRVPGSWEIPVAAGELARKEDIDAVIAIGVLIRGATPHFDYIASEVSKGLADLSLELRKPITFGVITADTLEQAIERAGTKHGNKGWEAALSAIEMANLFKSLRGGSGGSGGSGGSGGGDTITLPCRPAPPPHCSSNITGLILTRQGGYSNDNTVIFRPSGGDWRDIARCQIAGNVTSTQLFLNGSLAGNGTVIRSEDWRDNAKSICVQLNTSVEINCTGAGHCNISRAKWNNTLKQIASKLREQYGNKTIIFKPSSGGDPEFVNHSFNCGNVTFYCDSTQLFNSTWFNST

SEQ ID NO: 111 - protein, 365 aa, Artificial sequence
  recombinant gp120 lumazine synthase fusion protein
MPMGSLQPLATLYLLGMLVASVLAMQIYEGKLTAEGLRFGIVASRFNHALVDRLVEGAIDAIVRHGGREEDITLVRVPGSWEIPVAAGELARKEDIDAVIAIGVLIRGATPHFDYIASEVSKGLADLSLELRKPITFGVITADTLEQAIERAGTKHGNKGWEAALSAIEMANLFKSLRGGSGGSGGSGGSGGGDTITLPCRPAPPPHCSSNITGLILTRQGGYSNDNTVIFRPSGGDWRDIARCQIAGNVTSTQLFLNGSLAGGEVNGTSEDWRDNAKSICVQLNTSVEINCTGAGHCNISRAKWNNTLKQIASKLREQYGNKTIIFKPSSGGDPEFVNHSFNCGNVTFYCDSTQLFNSTWFNST

SEQ ID NO: 112 - protein, 366 aa, Artificial sequence
  recombinant gp120 lumazine synthase fusion protein
MPMGSLQPLATLYLLGMLVASVLAMQIYEGKLTAEGLRFGIVASRFNHALVDRLVEGAIDAIVRHGGREEDITLVRVPGSWEIPVAAGELARKEDIDAVIAIGVLIRGATPHFDYIASEVSKGLADLSLELRKPITFGVITADTLEQAIERAGTKHGNKGWEAALSAIEMANLFKSLRGGSGGSGGSGGSGGGDTITLPCNGTGPPPHCSSNITGLILTRQGGYSNDNTVIFRPSGGDWRDIARCQIAGNVTSTQLFLNGSLANGTVNGTSEDWRDNAKSICVQLNTSVEINCTGAGHCNISRAKWNNTLKQIASKLREQYGNKTIIFKPSSGGDPEFVNHSFNCGNVTFYCDSTQLFNSTWFNST

SEQ ID NO: 113 - protein, 365 aa, Artificial sequence
  recombinant gp120 lumazine synthase fusion protein
MPMGSLQPLATLYLLGMLVASVLAMQIYEGKLTAEGLRFGIVASRFNHALVDRLVEGAIDAIVRHGGREEDITLVRVPGSWEIPVAAGELARKEDIDAVIAIGVLIRGATPHFDYIASEVSKGLADLSLELRKPITFGVITADTLEQAIERAGTKHGNKGWEAALSAIEMANLFKSLRGGSGGSGGSGGSGGGDTITLPCRPAPPPNCTSNITGLILTRQGGYSNDNTVIFRPSGGDWRDIARCQIAGTVVSTQLFLNGSLAGNGTVIRSEDWRDNAKSICVQLNTSVEINCTGNGTCNISRAKWNNTLKQIASKLREQYGNKTIIFKPSSGGDPEFVNHSFNCGNVTFYCDSTQLFNSTWFNST